European Patent Specification EP 3 485 010 B1, published November 6, 2024. Title: POLYPEPTIDE VARIANTS. Applicant: Novozymes A/S. The sequence listing filed with the application follows.

SEQUENCE LISTING (26 sequences)

SEQ ID NO: 1 - protein, 182 aa, Bacillus cibi [sequence omitted]

SEQ ID NO: 2 - protein, 182 aa, Bacillus horikoshii
LPPGTPTKSEAQNQLNSLTVKSEGSMTGYSRDLFPHWSGQGNGCDTRQIVLQRDADYYTGTCPTTSGKWYSYFDGVIVYSPSEIDIDHIVPLAEAWRSGASSWTTEQRRAFANDLNGPQLIAVTASVNRSKGDQDPSTWQPPRAGARCAYAKWWINTKHRWNLHLQSSEKSSLQTMLNGCAY

SEQ ID NO: 3 - protein, 182 aa, Bacillus sp-62520
LPPGTPSKSEAQSQLNALTVKPEDPMTGYSRDHFPHWISQGNGCNTRQIVLQRDADYYSGACPVTTGKWYSYFDGVIVYSPSEIDIDHIVPLAEAWRSGASSWTTEKRRSFANDLNGPQLIAVTASVNRSKGDQDPSTWQPPRAGARCAYAKWWINTKHRWGLHLQSSEKSSLQSMLNGCAY

SEQ ID NO: 4 - protein, 182 aa, Bacillus horikoshii
LPPGTPSKSEAQSQLNSLTVKSEDPMTGYSRDHFPHWSGQGNGCDTRQIVLQRDADYYSGNCPVTSGKWYSYFDGVIVYSPSEIDIDHVVPLAEAWRSGASSWTTEQRRSFANDLNGPQLIAVTASVNRSKGDQDPSTWQPPRAGARCAYAKWWINTKHRWNLHLQSSEKSALQTMLNGCVY

SEQ ID NO: 5 - protein, 182 aa, Bacillus horikoshii
LPPGTPSKSEAQSQLNSLTVKTEDPMTGYSRDLFPHWSGQGSGCDTRQIVLQRDADYFTGTCPTTSGKWYSYFDGVIVYSPSEIDVDHIVPLAEAWRSGASSWTTEQRRAFANDLTGPQLIAVTASVNRSKGDQDPSTWQPPRAGARCAYAKWWINTKHRWNLHLQSSEKSSLQTMLNGCAY

SEQ ID NO: 6 - protein, 182 aa, Bacillus sp-16840
LPPGTPSKSEAQSQLNALTVKAEDPMTGYSRNLFPHWNSQGNGCNTRQLVLQRDADYYSGNCPVTSGRWYSYFDGVVVTSPSEIDIDHIVPLAEAWRSGASSWTTEKRKEFANDLNGPQLIAVTASVNRSKGDQDPSTWQPPRAAARCGYAKWWINTKYRWDLSLQSSEKSSLQTMLNTCSY

SEQ ID NO: 7 - protein, 182 aa, Bacillus sp-16840
LPPGTPSKSQAQSQLNALTVKAEDPMTGYSRNLFPHWSSQGNGCNTRQLVLQRDADYYSGNCPVTSGRWYSYFDGVVVTSPSEIDIDHIVPLAEAWRSGASSWTTEKRREFANDLNGPQLIAVTASVNRSKGDQDPSTWQPPRVAARCGYAKWWINTKYRWDLSLQSSEKSSLQTMLNTCSY

SEQ ID NO: 8 - protein, 182 aa, Bacillus sp-62668
LPPGTPSKSEAQSQLTSLTVKPEDPMTGYSRDHFPHWISQGNGCNTRQIVLQRDADYYSGNCPVTTGKWYSYFDGVIVYSPSEIDIDHIVPLAEAWRSGASSWTAEQRRNFANDLNGPQLIAVTASVNRSKGDQDPSTWQPPRTGARCAYAKWWINTKYRWGLHLQSSEKSSLQSMLNGCAY

SEQ ID NO: 9 - protein, 185 aa, Bacillus sp-13395
ASAFPPGTPSKSTAQSQLNSLPVKSEGSMNGYSRDKFPHWISQGDGCDTRQLVLKRDGDYYSGSCPVTSGKWYSYYDGITVYSPSEIDIDHIVPLAEAWRSGASGWTTEKRQSFANDLNGPQLIAVTASVNRSKGDQDPSTWQPPRSGSHCAYAKMWVNTKYRWGLHLQSAEKSALQSMLNACSY

SEQ ID NO: 10 - protein, 185 aa, Bacillus horneckiae
ASAFPPGTPSKSTAQSQLNSLTVKSEGSMTGYSRDKFPHWISQGDGCDTRQLVLKRDGDYYSGNCPVTSGKWYSYYDGITVYSPSEIDIDHIVPLAEAWRSGASGWTTEKRQSFANDLNGPQLIAVTASVNRSKGDQDPSTWQPPRSGSHCAYAKMWVNTKYRWGLHVQSAEKSALQSMLNACSY

SEQ ID NO: 11 - protein, 182 aa, Bacillus sp-11238
FPPEIPSKSTAQSQLNSLTVKSEDAMTGYSRDKFPHWISQGDGCDTRQMVLKRDADYYSGSCPVTSGKWYSYYDGITVYSPSEIDIDHIVPLAEAWRSGASSWTTEKRRNFANDLNGPQLIAVTASVNRSKGDQDPSTWQPPRSGARCAYAKMWVNTKYRWGLHLQSAEKSGLESMLNTCSY

SEQ ID NO: 12 - protein, 182 aa, Bacillus SP-62451
LPPDLPSKSTTQAQLNSLNVKNEESMSGYSREKFPHWISQGDGCDTRQVILKRDADNYSGNCPVTSGKWYSYYDGITFNDPSQLDIDHVVPLAEAWRSGASSWSTAKREDFANDLNGPQLIAVSASSNRSKGDQDPSTWQPPRAGANCAYAKMWINTKYNWGLHLQSSEKTALQGMLNSCSY

SEQ ID NO: 13 - protein, 182 aa, Bacillus sp-18318
FPPGTPSKSTAQSQLNSLTVKSEGSMTGYSRDKFPHWIGQGSGCDTRQLVLQRDADYYSGSCPVTSGKWYSYYDGVTFYDPSDLDIDHVVPLAEAWRSGASSWSTQKRKDFANDLSGPQLIAVSASSNRSKGDQDPSTWQPTRSGAACGYSKWWISTKHKWGLSLQSSEKNALQGMLNSCVY

SEQ ID NO: 14 - protein, 182 aa, Bacillus idriensis
LPPGTPSKSTAQSQLNALTVQTEGSMTGYSRDKFPHWISQGNGCDTRQVVLQRDADYYSGTCPVTSGKWYSYYDGVTLYNPSDLDIDHVVALAEAWRSGASSWTTDKREDFANDLSGTQLIAVSASTNRSKGDQDPSTWQPPRSGAACGYAKWWISTKYKWNLNLQSSEKTALQSMLNSCSY

SEQ ID NO: 15 - protein, 182 aa, Bacillus algicola
FPPGTPSKSEAQSQLNSLTVQSEGSMSGYSRDKFPHWIGQGNGCDTRQLVLQRDADYYSGDCPVTSGKWYSYFDGVTVYDPSDLDIDHMVPMAEAWRSGASSWSTQKREDFANDLSGPHLIAVTASSNRSKGDQDPSTWKPTRYGAHCGYAKWWINTKYVYDLTLQSSEKTELQSMLNTCSY

SEQ ID NO: 16 - protein, 182 aa, Enviromental sample J
LPPNIPSKADALTKLNALTVQTEGPMTGYSRDLFPHWSSQGNGCNTRHVVLKRDADSVVDTCPVTTGRWYSYYDGLVFTSASDIDIDHVVPLAEAWRSGASSWTSTKRQSFANDLNGPQLIAVSATSNRSKGDQDPSTWQPPRAGARCAYAKMWVETKSRWGLTLQSSEKAALQTAINACSY

SEQ ID NO: 17 - protein, 182 aa, Bacillus vietnamensis
FPPGTPSKSTAQSQLNALTVKSESSMTGYSRDKFPHWIGQRNGCDTRQLVLQRDADSYSGSCPVTSGSWYSYYDGVTFTDPSDLDIDHVVPLAEAWRSGASSWTTAKREDFANDLSGPQLIAVSASSNRSKGDQDPSTWQPPRSGAACGYSKWWISTKYKWGLSLQSSEKTALQGMLNSCIY

SEQ ID NO: 18 - protein, 182 aa, Bacillus hwajinpoensis
IPPGTPSKSAAQSQLDSLAVQSEGSMSGYSRDKFPHWIGQGNGCDTRQLVLQRDADYYSGDCPVTSGKWYSYFDGVQVYDPSYLDIDHMVPLAEAWRSGASSWSTQKREDFANDLDGPHLIAVTASSNRSKGDQDPSTWKPTRYSAHCGYAKWWINTKYVYDLNLQSSEKSALQSMLNTCSY

SEQ ID NO: 19 - protein, 182 aa, Paenibacillus mucilaginosus
LPPGTPSKSTAQSQLNSLTVKSESTMTGYSRDKFPHWTSQGGGCDTRQVVLKRDADYYSGSCPVTSGKWYSYYDGITVYSPSEIDIDHIVPLAEAWRSGASSWTTEKRQNFANDLGGPQLIAVTASSNRAKGDQDPSTWKPTRSGAHCAYAKWWINTKYRWGLHLQSSEKTALQSMLNTCSY

SEQ ID NO: 20 - protein, 182 aa, Bacillus indicus
TPPGTPSKSTAQTQLNALTVKTEGSMTGYSRDLFPHWISQGSGCDTRQVVLKRDADYYSGSCPVTSGKWYSYYDGVTFYDPSDLDIDHIVPLAEAWRSGASSWTTSKRQDFANDLSGPQLIAVSASTNRSKGDQDPSTWQPPRAGAACGYSKWWISTKYKWGLSLQSSEKTALQGMLNSCSY

SEQ ID NO: 21 - protein, 182 aa, Bacillus marisflavi
TPPVTPSKATSQSQLNGLTVKTEGAMTGYSRDKFPHWSSQGGGCDTRQVVLKRDADSYSGNCPVTSGSWYSYYDGVKFTNPSDLDIDHIVPLAEAWRSGASSWTTAQREAFANDLSGSQLIAVSASSNRSKGDQDPSTWQPPRAGAKCGYAKWWISTKSKWNLSLQSSEKTALQGMLNSCVY

SEQ ID NO: 22 - protein, 184 aa, Bacillus luciferensis
ASLPPGIPSLSTAQSQLNSLTVKSEGSLTGYSRDVFPHWISQGSGCDTRQVVLKRDADYYSGNCPVTSGKWYSYYDGVTVYSPSEIDIDHVVPLAEAWRSGASSWTTEKRQNFANDLNGPQLIAVTASSNRSKGDQDPSTWQPTRTGARCAYAKMWINTKYRWGLHLQSSEKSALQSMLNTCSY

SEQ ID NO: 23 - protein, 182 aa, Bacillus marisflavi
TPPVTPSKETSQSQLNGLTVKTEGAMTGYSRDKFPHWSSQGGGCDTRQVVLKRDADSYSGNCPVTSGSWYSYYDGVKFTHPSDLDIDHIVPLAEAWRSGASSWTTAQREAFANDLSGSQLIAVSASSNRSKGDQDPSTWQPPRAGAKCGYAKWWISTKSKWNLSLQSSEKTALQGMLNSCVY

SEQ ID NO: 24 - protein, 182 aa, Bacillus sp. SA2-6
LPSGIPSKSTAQSQLNSLTVKSEGSMTGYSRDKFPHWISQGGGCDTRQVVLKRDADYYSGNCPVTSGKWYSYYDGISVYSPSEIDIDHVVPLAEAWRSGASSWTTTKRQNFANDLNGPQLIAVTASVNRSKGDQDPSTWQPPRYGARCAYAKMWINTKYRWDLNLQSSEKSSLQSMLDTCSY

SEQ ID NO: 25 - protein, 7 aa, Artificial
  Motif
  MISC_FEATURE (1)..(1): Xaa = Asp (D) or Met (M) or Leu (L)
  MISC_FEATURE (2)..(2): Xaa = Ser (S) or Thr (T)
  MISC_FEATURE (7)..(7): Xaa = Asp (D) or Asn (N)
XXGYSRX

SEQ ID NO: 26 - protein, 8 aa, Artificial
  Motif
  MISC_FEATURE (3)..(3): Xaa = any amino acid
ASXNRSKG